European Patent Application EP 4 212 543 A1, published July 19, 2023. Title: Fusion Protein comprising a Receptor Binding Domain Derived From Coronavirus and Nucleocapsid Protein, and Uses Thereof. Applicant: GI Cell, Inc. The sequence listing filed with the application follows.

SEQUENCE LISTING (26 sequences)

SEQ ID NO: 1 - protein, 219 aa, Artificial Sequence
  Wild type RBD
RVQPTESIVRFPNITNLCPFGEVFNATRFASVYAWNRKRISNCVADYSVLYNSASFSTFKCYGVSPTKLNDLCFTNVYADSFVIRGDEVRQIAPGQTGKIADYNYKLPDDFTGCVIAWNSNNLDSKVGGNYNYLYRLFRKSNLKPFERDISTEIYQAGSTPCNGVEGFNCYFPLQSYGFQPTNGVGYQPYRVVVLSFELLHAPATVCGPKKSTNLVKNK

SEQ ID NO: 2 - protein, 231 aa, Artificial Sequence
  IgG1 Fc domain
EPKSSDKTHTCPPCPAPELLGGPSVFLFPPKPKDTLMISRTPEVTCVVVDVSHEDPEVKFNWYVDGVEVHNAKTKPREEQYNSTYRVVSVLTVLHQDWLNGKEYKCKVSNKALPAPIEKTISKAKGQPREPQVYTLPPSRDELTKNQVSLTCLVKGFYPSDIAVEWESNGQPENNYKTTPPVLDSDGSFFLYSKLTVDKSRWQQGNVFSCSVMHEALHNHYTQKSLSLSPG

SEQ ID NO: 3 - protein, 419 aa, Artificial Sequence
  N protein_full
MSDNGPQNQRNAPRITFGGPSDSTGSNQNGERSGARSKQRRPQGLPNNTASWFTALTQHGKEDLKFPRGQGVPINTNSSPDDQIGYYRRATRRIRGGDGKMKDLSPRWYFYYLGTGPEAGLPYGANKDGIIWVATEGALNTPKDHIGTRNPANNAAIVLQLPQGTTLPKGFYAEGSRGGSQASSRSSSRSRNSSRNSTPGSSRGTSPARMAGNGGDAALALLLLDRLNQLESKMSGKGQQQQGQTVTKKSAAEASKKPRQKRTATKAYNVTQAFGRRGPEQTQGNFGDQELIRQGTDYKHWPQIAQFAPSASAFFGMSRIGMEVTPSGTWLTYTGAIKLDDKDPNFKDQVILLNKHIDAYKTFPPTEPKKDKKKKADETQALPQRQKKQQTVTLLPAADLDDFSKQLQQSMSSADSTQA

SEQ ID NO: 4 - protein, 156 aa, Artificial Sequence
  N protein_RNA binding domain
RSKQRRPQGLPNNTASWFTALTQHGKEDLKFPRGQGVPINTNSSPDDQIGYYRRATRRIRGGDGKMKDLSPRWYFYYLGTGPEAGLPYGANKDGIIWVATEGALNTPKDHIGTRNPANNAAIVLQLPQGTTLPKGFYAEGSRGGSQASSRSSSRSR

SEQ ID NO: 5 - protein, 15 aa, Artificial Sequence
  Linker1
GGGGSGGGGSGGGGS

SEQ ID NO: 6 - protein, 20 aa, Artificial Sequence
  Linker2
GGGGSGGGGSGGGGSGGGGS

SEQ ID NO: 7 - protein, 18 aa, Artificial Sequence
  Signal peptide
MKWVTFISLLFLFSSAYS

SEQ ID NO: 8 - DNA, 657 bp, Artificial Sequence
  Wild type RBD_DNA sequence
agagttcagcctaccgagtccatcgtgcggttccccaacatcaccaacctgtgtcctttcggcgaggtgttcaacgctaccagattcgcctctgtgtacgcctggaaccggaagcggatctctaactgcgtggccgactactccgtgctgtacaactctgcctccttcagcaccttcaagtgctacggcgtgtcccctaccaagctgaacgacctgtgcttcaccaacgtgtacgccgactccttcgtgatcaggggcgacgaagttcggcagatcgctcctggacagaccggcaagatcgccgactacaattacaagctgcccgacgacttcaccggctgcgtgatcgcttggaactccaacaacctggactccaaagtcggcggcaactacaactacctgtaccggctgttccggaagtccaacctgaagcctttcgagcgggacatctccaccgagatctaccaggctggcagcaccccttgcaatggcgtcgagggcttcaactgctacttcccactgcagtcctacggcttccagcctaccaatggcgtgggctaccagccttatagagtggtggtgctgtccttcgagctgctgcatgctcctgctaccgtgtgcggccctaagaaatctaccaacctggtcaagaacaag

SEQ ID NO: 9 - DNA, 693 bp, Artificial Sequence
  IgG1 Fc domain_DNA sequence
gaacctaagtcctccgacaagacccacacctgtcctccatgtcctgctccagaactgctcggcggaccttccgtgtttctgttcccacctaagccaaaggacaccctgatgatcagcagaacccctgaagtgacctgcgtggtggtggatgtgtctcacgaggaccccgaagtgaagttcaattggtacgtggacggcgtggaagtgcacaacgccaagaccaagcctagagaggaacagtacaactccacctacagagtggtgtccgtgctgaccgtgctgcaccaggattggctgaacggcaaagagtacaagtgcaaggtgtccaacaaggccctgcctgctcctatcgaaaagaccatctccaaggccaagggccagcctagggaaccccaggtttacacactgcctccatctcgggacgagctgaccaagaatcaggtgtccctgacctgtctggtcaagggcttctacccttccgatatcgccgtggaatgggagagcaatggccagcctgagaacaactacaagacaacccctcctgtgctggactccgacggctcattcttcctgtatagcaagctgacagtggacaagtcccggtggcagcagggcaacgtgttctcctgttctgtgatgcacgaggccctgcacaaccactacacccagaagagtctgtccttgagcccgggc

SEQ ID NO: 10 - DNA, 1260 bp, Artificial Sequence
  N protein_Full DNA sequence
atgtctgataatggaccccaaaatcagcgaaatgcaccccgcattacgtttggtggaccctcagattcaactggcagtaaccagaatggagaacgcagtggggcgcgatcaaaacaacgtcggccccaaggtttacccaataatactgcgtcttggttcaccgctctcactcaacatggcaaggaagaccttaaattccctcgaggacaaggcgttccaattaacaccaatagcagtccagatgaccaaattggctactaccgaagagctaccagacgaattcgtggtggtgacggtaaaatgaaagatctcagtccaagatggtatttctactacctaggaactgggccagaagctggacttccctatggtgctaacaaagacggcatcatatgggttgcaactgagggagccttgaatacaccaaaagatcacattggcacccgcaatcctgctaacaatgctgcaatcgtgctacaacttcctcaaggaacaacattgccaaaaggcttctacgcagaagggagcagaggcggcagtcaagcctcttctcgttcctcatcacgtagtcgcaacagttcaagaaattcaactccaggcagcagtaggggaacttctcctgctagaatggctggcaatggcggtgatgctgctcttgctttgctgctgcttgacagattgaaccagcttgagagcaaaatgtctggtaaaggccaacaacaacaaggccaaactgtcactaagaaatctgctgctgaggcttctaagaagcctcggcaaaaacgtactgccactaaagcatacaatgtaacacaagctttcggcagacgtggtccagaacaaacccaaggaaattttggggaccaggaactaatcagacaaggaactgattacaaacattggccgcaaattgcacaatttgcccccagcgcttcagcgttcttcggaatgtcgcgcattggcatggaagtcacaccttcgggaacgtggttgacctacacaggtgccatcaaattggatgacaaagatccaaatttcaaagatcaagtcattttgctgaataagcatattgacgcatacaaaacattcccaccaacagagcctaaaaaggacaaaaagaagaaggctgatgaaactcaagccttaccgcagagacagaagaaacagcaaactgtgactcttcttcctgctgcagatttggatgatttctccaaacaattgcaacaatccatgagcagtgctgactcaactcaggcctaa

SEQ ID NO: 11 - DNA, 468 bp, Artificial Sequence
  N protein_RNA binding domain_DNA sequence
cggtctaagcagagaaggcctcagggcctgcctaacaataccgcctcctggtttaccgctctgacccagcacggcaaagaggacctgaagttccctagaggacagggcgtgcccatcaacaccaactctagccctgacgaccagatcggctactacagacgggccaccagaagaatcagaggcggcgacggcaagatgaaggacctgtctcctcggtggtacttctactacctcggcaccggaccagaggctggattgccttatggcgccaacaaggacggcatcatctgggttgcaacagagggcgctctgaacacccctaaggaccacatcggcacccggaatcctgccaacaatgctgccattgtgctgcagctgccacagggcacaacactgcctaagggcttttacgccgagggctctagaggcggctctcaggcctcttccagatcctccagtagatcacgt

SEQ ID NO: 12 - DNA, 45 bp, Artificial Sequence
  Linker1_DNA sequence
ggcggcggaggatccggcggtggtggttccggcggaggcggttct

SEQ ID NO: 13 - DNA, 60 bp, Artificial Sequence
  Linker2_DNA sequence
ggtggcggcggttcaggcggcggtggaagtggcggtggcggatctggcggaggtggtagt

SEQ ID NO: 14 - DNA, 54 bp, Artificial Sequence
  Signal peptide_DNA sequence
atgaaatgggtcacctttatctccctgctgttcctgttctcctccgcctactct

SEQ ID NO: 15 - protein, 246 aa, Artificial Sequence
  Fusion protein_IgG1 Fc
GGGGSGGGGSGGGGSEPKSSDKTHTCPPCPAPELLGGPSVFLFPPKPKDTLMISRTPEVTCVVVDVSHEDPEVKFNWYVDGVEVHNAKTKPREEQYNSTYRVVSVLTVLHQDWLNGKEYKCKVSNKALPAPIEKTISKAKGQPREPQVYTLPPSRDELTKNQVSLTCLVKGFYPSDIAVEWESNGQPENNYKTTPPVLDSDGSFFLYSKLTVDKSRWQQGNVFSCSVMHEALHNHYTQKSLSLSPG

SEQ ID NO: 16 - protein, 465 aa, Artificial Sequence
  Fusion protein_RBDwt-Fc
RVQPTESIVRFPNITNLCPFGEVFNATRFASVYAWNRKRISNCVADYSVLYNSASFSTFKCYGVSPTKLNDLCFTNVYADSFVIRGDEVRQIAPGQTGKIADYNYKLPDDFTGCVIAWNSNNLDSKVGGNYNYLYRLFRKSNLKPFERDISTEIYQAGSTPCNGVEGFNCYFPLQSYGFQPTNGVGYQPYRVVVLSFELLHAPATVCGPKKSTNLVKNKGGGGSGGGGSGGGGSEPKSSDKTHTCPPCPAPELLGGPSVFLFPPKPKDTLMISRTPEVTCVVVDVSHEDPEVKFNWYVDGVEVHNAKTKPREEQYNSTYRVVSVLTVLHQDWLNGKEYKCKVSNKALPAPIEKTISKAKGQPREPQVYTLPPSRDELTKNQVSLTCLVKGFYPSDIAVEWESNGQPENNYKTTPPVLDSDGSFFLYSKLTVDKSRWQQGNVFSCSVMHEALHNHYTQKSLSLSPG

SEQ ID NO: 17 - protein, 485 aa, Artificial Sequence
  Fusion protein_Fc-RBDwt
GGGGSGGGGSGGGGSEPKSSDKTHTCPPCPAPELLGGPSVFLFPPKPKDTLMISRTPEVTCVVVDVSHEDPEVKFNWYVDGVEVHNAKTKPREEQYNSTYRVVSVLTVLHQDWLNGKEYKCKVSNKALPAPIEKTISKAKGQPREPQVYTLPPSRDELTKNQVSLTCLVKGFYPSDIAVEWESNGQPENNYKTTPPVLDSDGSFFLYSKLTVDKSRWQQGNVFSCSVMHEALHNHYTQKSLSLSPGGGGGSGGGGSGGGGSGGGGSRVQPTESIVRFPNITNLCPFGEVFNATRFASVYAWNRKRISNCVADYSVLYNSASFSTFKCYGVSPTKLNDLCFTNVYADSFVIRGDEVRQIAPGQTGKIADYNYKLPDDFTGCVIAWNSNNLDSKVGGNYNYLYRLFRKSNLKPFERDISTEIYQAGSTPCNGVEGFNCYFPLQSYGFQPTNGVGYQPYRVVVLSFELLHAPATVCGPKKSTNLVKNK

SEQ ID NO: 18 - protein, 402 aa, Artificial Sequence
  Fusion protein_N-Fc
RSKQRRPQGLPNNTASWFTALTQHGKEDLKFPRGQGVPINTNSSPDDQIGYYRRATRRIRGGDGKMKDLSPRWYFYYLGTGPEAGLPYGANKDGIIWVATEGALNTPKDHIGTRNPANNAAIVLQLPQGTTLPKGFYAEGSRGGSQASSRSSSRSRGGGGSGGGGSGGGGSEPKSSDKTHTCPPCPAPELLGGPSVFLFPPKPKDTLMISRTPEVTCVVVDVSHEDPEVKFNWYVDGVEVHNAKTKPREEQYNSTYRVVSVLTVLHQDWLNGKEYKCKVSNKALPAPIEKTISKAKGQPREPQVYTLPPSRDELTKNQVSLTCLVKGFYPSDIAVEWESNGQPENNYKTTPPVLDSDGSFFLYSKLTVDKSRWQQGNVFSCSVMHEALHNHYTQKSLSLSPG

SEQ ID NO: 19 - protein, 641 aa, Artificial Sequence
  Fusion protein_GIC-1114
RSKQRRPQGLPNNTASWFTALTQHGKEDLKFPRGQGVPINTNSSPDDQIGYYRRATRRIRGGDGKMKDLSPRWYFYYLGTGPEAGLPYGANKDGIIWVATEGALNTPKDHIGTRNPANNAAIVLQLPQGTTLPKGFYAEGSRGGSQASSRSSSRSRGGGGSGGGGSGGGGSEPKSSDKTHTCPPCPAPELLGGPSVFLFPPKPKDTLMISRTPEVTCVVVDVSHEDPEVKFNWYVDGVEVHNAKTKPREEQYNSTYRVVSVLTVLHQDWLNGKEYKCKVSNKALPAPIEKTISKAKGQPREPQVYTLPPSRDELTKNQVSLTCLVKGFYPSDIAVEWESNGQPENNYKTTPPVLDSDGSFFLYSKLTVDKSRWQQGNVFSCSVMHEALHNHYTQKSLSLSPGGGGGSGGGGSGGGGSGGGGSRVQPTESIVRFPNITNLCPFGEVFNATRFASVYAWNRKRISNCVADYSVLYNSASFSTFKCYGVSPTKLNDLCFTNVYADSFVIRGDEVRQIAPGQTGKIADYNYKLPDDFTGCVIAWNSNNLDSKVGGNYNYLYRLFRKSNLKPFERDISTEIYQAGSTPCNGVEGFNCYFPLQSYGFQPTNGVGYQPYRVVVLSFELLHAPATVCGPKKSTNLVKNK

SEQ ID NO: 20 - protein, 641 aa, Artificial Sequence
  Fusion protein_GIC-1114N
RVQPTESIVRFPNITNLCPFGEVFNATRFASVYAWNRKRISNCVADYSVLYNSASFSTFKCYGVSPTKLNDLCFTNVYADSFVIRGDEVRQIAPGQTGKIADYNYKLPDDFTGCVIAWNSNNLDSKVGGNYNYLYRLFRKSNLKPFERDISTEIYQAGSTPCNGVEGFNCYFPLQSYGFQPTNGVGYQPYRVVVLSFELLHAPATVCGPKKSTNLVKNKGGGGSGGGGSGGGGSEPKSSDKTHTCPPCPAPELLGGPSVFLFPPKPKDTLMISRTPEVTCVVVDVSHEDPEVKFNWYVDGVEVHNAKTKPREEQYNSTYRVVSVLTVLHQDWLNGKEYKCKVSNKALPAPIEKTISKAKGQPREPQVYTLPPSRDELTKNQVSLTCLVKGFYPSDIAVEWESNGQPENNYKTTPPVLDSDGSFFLYSKLTVDKSRWQQGNVFSCSVMHEALHNHYTQKSLSLSPGGGGGSGGGGSGGGGSGGGGSRSKQRRPQGLPNNTASWFTALTQHGKEDLKFPRGQGVPINTNSSPDDQIGYYRRATRRIRGGDGKMKDLSPRWYFYYLGTGPEAGLPYGANKDGIIWVATEGALNTPKDHIGTRNPANNAAIVLQLPQGTTLPKGFYAEGSRGGSQASSRSSSRSR

SEQ ID NO: 21 - DNA, 738 bp, Artificial Sequence
  Fusion protein_DNA sequence_IgG1 Fc
ggcggcggaggatccggcggtggtggttccggcggaggcggttctgaacctaagtcctccgacaagacccacacctgtcctccatgtcctgctccagaactgctcggcggaccttccgtgtttctgttcccacctaagccaaaggacaccctgatgatcagcagaacccctgaagtgacctgcgtggtggtggatgtgtctcacgaggaccccgaagtgaagttcaattggtacgtggacggcgtggaagtgcacaacgccaagaccaagcctagagaggaacagtacaactccacctacagagtggtgtccgtgctgaccgtgctgcaccaggattggctgaacggcaaagagtacaagtgcaaggtgtccaacaaggccctgcctgctcctatcgaaaagaccatctccaaggccaagggccagcctagggaaccccaggtttacacactgcctccatctcgggacgagctgaccaagaatcaggtgtccctgacctgtctggtcaagggcttctacccttccgatatcgccgtggaatgggagagcaatggccagcctgagaacaactacaagacaacccctcctgtgctggactccgacggctcattcttcctgtatagcaagctgacagtggacaagtcccggtggcagcagggcaacgtgttctcctgttctgtgatgcacgaggccctgcacaaccactacacccagaagagtctgtccttgagcccgggc

SEQ ID NO: 22 - DNA, 1395 bp, Artificial Sequence
  Fusion protein_DNA sequence_RBDwt-Fc
agagttcagcctaccgagtccatcgtgcggttccccaacatcaccaacctgtgtcctttcggcgaggtgttcaacgctaccagattcgcctctgtgtacgcctggaaccggaagcggatctctaactgcgtggccgactactccgtgctgtacaactctgcctccttcagcaccttcaagtgctacggcgtgtcccctaccaagctgaacgacctgtgcttcaccaacgtgtacgccgactccttcgtgatcaggggcgacgaagttcggcagatcgctcctggacagaccggcaagatcgccgactacaattacaagctgcccgacgacttcaccggctgcgtgatcgcttggaactccaacaacctggactccaaagtcggcggcaactacaactacctgtaccggctgttccggaagtccaacctgaagcctttcgagcgggacatctccaccgagatctaccaggctggcagcaccccttgcaatggcgtcgagggcttcaactgctacttcccactgcagtcctacggcttccagcctaccaatggcgtgggctaccagccttatagagtggtggtgctgtccttcgagctgctgcatgctcctgctaccgtgtgcggccctaagaaatctaccaacctggtcaagaacaagggcggcggaggatccggcggtggtggttccggcggaggcggttctgaacctaagtcctccgacaagacccacacctgtcctccatgtcctgctccagaactgctcggcggaccttccgtgtttctgttcccacctaagccaaaggacaccctgatgatcagcagaacccctgaagtgacctgcgtggtggtggatgtgtctcacgaggaccccgaagtgaagttcaattggtacgtggacggcgtggaagtgcacaacgccaagaccaagcctagagaggaacagtacaactccacctacagagtggtgtccgtgctgaccgtgctgcaccaggattggctgaacggcaaagagtacaagtgcaaggtgtccaacaaggccctgcctgctcctatcgaaaagaccatctccaaggccaagggccagcctagggaaccccaggtttacacactgcctccatctcgggacgagctgaccaagaatcaggtgtccctgacctgtctggtcaagggcttctacccttccgatatcgccgtggaatgggagagcaatggccagcctgagaacaactacaagacaacccctcctgtgctggactccgacggctcattcttcctgtatagcaagctgacagtggacaagtcccggtggcagcagggcaacgtgttctcctgttctgtgatgcacgaggccctgcacaaccactacacccagaagagtctgtccttgagcccgggc

SEQ ID NO: 23 - DNA, 1455 bp, Artificial Sequence
  Fusion protein_DNA sequence_Fc-RBDwt
ggcggcggaggatccggcggtggtggttccggcggaggcggttctgaacctaagtcctccgacaagacccacacctgtcctccatgtcctgctccagaactgctcggcggaccttccgtgtttctgttcccacctaagccaaaggacaccctgatgatcagcagaacccctgaagtgacctgcgtggtggtggatgtgtctcacgaggaccccgaagtgaagttcaattggtacgtggacggcgtggaagtgcacaacgccaagaccaagcctagagaggaacagtacaactccacctacagagtggtgtccgtgctgaccgtgctgcaccaggattggctgaacggcaaagagtacaagtgcaaggtgtccaacaaggccctgcctgctcctatcgaaaagaccatctccaaggccaagggccagcctagggaaccccaggtttacacactgcctccatctcgggacgagctgaccaagaatcaggtgtccctgacctgtctggtcaagggcttctacccttccgatatcgccgtggaatgggagagcaatggccagcctgagaacaactacaagacaacccctcctgtgctggactccgacggctcattcttcctgtatagcaagctgacagtggacaagtcccggtggcagcagggcaacgtgttctcctgttctgtgatgcacgaggccctgcacaaccactacacccagaagagtctgtccttgagcccgggcggtggcggcggttcaggcggcggtggaagtggcggtggcggatctggcggaggtggtagtagagttcagcctaccgagtccatcgtgcggttccccaacatcaccaacctgtgtcctttcggcgaggtgttcaacgctaccagattcgcctctgtgtacgcctggaaccggaagcggatctctaactgcgtggccgactactccgtgctgtacaactctgcctccttcagcaccttcaagtgctacggcgtgtcccctaccaagctgaacgacctgtgcttcaccaacgtgtacgccgactccttcgtgatcaggggcgacgaagttcggcagatcgctcctggacagaccggcaagatcgccgactacaattacaagctgcccgacgacttcaccggctgcgtgatcgcttggaactccaacaacctggactccaaagtcggcggcaactacaactacctgtaccggctgttccggaagtccaacctgaagcctttcgagcgggacatctccaccgagatctaccaggctggcagcaccccttgcaatggcgtcgagggcttcaactgctacttcccactgcagtcctacggcttccagcctaccaatggcgtgggctaccagccttatagagtggtggtgctgtccttcgagctgctgcatgctcctgctaccgtgtgcggccctaagaaatctaccaacctggtcaagaacaag

SEQ ID NO: 24 - DNA, 1206 bp, Artificial Sequence
  Fusion protein_DNA sequence_N-Fc
cggtctaagcagagaaggcctcagggcctgcctaacaataccgcctcctggtttaccgctctgacccagcacggcaaagaggacctgaagttccctagaggacagggcgtgcccatcaacaccaactctagccctgacgaccagatcggctactacagacgggccaccagaagaatcagaggcggcgacggcaagatgaaggacctgtctcctcggtggtacttctactacctcggcaccggaccagaggctggattgccttatggcgccaacaaggacggcatcatctgggttgcaacagagggcgctctgaacacccctaaggaccacatcggcacccggaatcctgccaacaatgctgccattgtgctgcagctgccacagggcacaacactgcctaagggcttttacgccgagggctctagaggcggctctcaggcctcttccagatcctccagtagatcacgtggcggcggaggatccggtggtggtggatctggtggcggaggctctgaacctaagtcctccgacaagacccacacctgtcctccatgtcctgctccagaactgctcggcggaccttccgtgtttctgttcccacctaagccaaaggacaccctgatgatcagcagaacccctgaagtgacctgcgtggtggtggatgtgtctcacgaggaccccgaagtgaagttcaattggtacgtggacggcgtggaagtgcacaacgccaagaccaagcctagagaggaacagtacaactccacctacagagtggtgtccgtgctgaccgtgctgcaccaggattggctgaacggcaaagagtacaagtgcaaggtgtccaacaaggccctgcctgctcctatcgaaaagaccatctccaaggccaagggccagcctagggaaccccaggtttacacactgcctccatctcgggacgagctgaccaagaatcaggtgtccctgacctgtctggtcaagggcttctacccttccgatatcgccgtggaatgggagagcaatggccagcctgagaacaactacaagacaacccctcctgtgctggactccgacggctcattcttcctgtatagcaagctgacagtggacaagtcccggtggcagcagggcaacgtgttctcctgttctgtgatgcacgaggccctgcacaaccactacacccagaagagtctgtccttgagcccgggc

SEQ ID NO: 25 - DNA, 1923 bp, Artificial Sequence
  Fusion protein_DNA sequence_GIC-1114
cggtctaagcagagaaggcctcagggcctgcctaacaataccgcctcctggtttaccgctctgacccagcacggcaaagaggacctgaagttccctagaggacagggcgtgcccatcaacaccaactctagccctgacgaccagatcggctactacagacgggccaccagaagaatcagaggcggcgacggcaagatgaaggacctgtctcctcggtggtacttctactacctcggcaccggaccagaggctggattgccttatggcgccaacaaggacggcatcatctgggttgcaacagagggcgctctgaacacccctaaggaccacatcggcacccggaatcctgccaacaatgctgccattgtgctgcagctgccacagggcacaacactgcctaagggcttttacgccgagggctctagaggcggctctcaggcctcttccagatcctccagtagatcacgtggcggcggaggatccggcggtggtggttccggcggaggcggttctgaacctaagtcctccgacaagacccacacctgtcctccatgtcctgctccagaactgctcggcggaccttccgtgtttctgttcccacctaagccaaaggacaccctgatgatcagcagaacccctgaagtgacctgcgtggtggtggatgtgtctcacgaggaccccgaagtgaagttcaattggtacgtggacggcgtggaagtgcacaacgccaagaccaagcctagagaggaacagtacaactccacctacagagtggtgtccgtgctgaccgtgctgcaccaggattggctgaacggcaaagagtacaagtgcaaggtgtccaacaaggccctgcctgctcctatcgaaaagaccatctccaaggccaagggccagcctagggaaccccaggtttacacactgcctccatctcgggacgagctgaccaagaatcaggtgtccctgacctgtctggtcaagggcttctacccttccgatatcgccgtggaatgggagagcaatggccagcctgagaacaactacaagacaacccctcctgtgctggactccgacggctcattcttcctgtatagcaagctgacagtggacaagtcccggtggcagcagggcaacgtgttctcctgttctgtgatgcacgaggccctgcacaaccactacacccagaagagtctgtccttgagcccgggcggtggcggtggaagcggaggtggcggatctggtggcggaggtagtggcggaggcggatctagagttcagcctaccgagtccatcgtgcggttccccaacatcaccaacctgtgtcctttcggcgaggtgttcaacgctaccagattcgcctctgtgtacgcctggaaccggaagcggatctctaactgcgtggccgactactccgtgctgtacaactctgcctccttcagcaccttcaagtgctacggcgtgtcccctaccaagctgaacgacctgtgcttcaccaacgtgtacgccgactccttcgtgatcaggggcgacgaagttcggcagatcgctcctggacagaccggcaagatcgccgactacaattacaagctgcccgacgacttcaccggctgcgtgatcgcttggaactccaacaacctggactccaaagtcggcggcaactacaactacctgtaccggctgttccggaagtccaacctgaagcctttcgagcgggacatctccaccgagatctaccaggctggcagcaccccttgcaatggcgtcgagggcttcaactgctacttcccactgcagtcctacggcttccagcctaccaatggcgtgggctaccagccttatagagtggtggtgctgtccttcgagctgctgcatgctcctgctaccgtgtgcggccctaagaaatctaccaacctggtcaagaacaag

SEQ ID NO: 26 - DNA, 1923 bp, Artificial Sequence
  Fusion protein_DNA sequence_GIC-1114N
agagttcagcctaccgagtccatcgtgcggttccccaacatcaccaacctgtgtcctttcggcgaggtgttcaacgctaccagattcgcctctgtgtacgcctggaaccggaagcggatctctaactgcgtggccgactactccgtgctgtacaactctgcctccttcagcaccttcaagtgctacggcgtgtcccctaccaagctgaacgacctgtgcttcaccaacgtgtacgccgactccttcgtgatcaggggcgacgaagttcggcagatcgctcctggacagaccggcaagatcgccgactacaattacaagctgcccgacgacttcaccggctgcgtgatcgcttggaactccaacaacctggactccaaagtcggcggcaactacaactacctgtaccggctgttccggaagtccaacctgaagcctttcgagcgggacatctccaccgagatctaccaggctggcagcaccccttgcaatggcgtcgagggcttcaactgctacttcccactgcagtcctacggcttccagcctaccaatggcgtgggctaccagccttatagagtggtggtgctgtccttcgagctgctgcatgctcctgctaccgtgtgcggccctaagaaatctaccaacctggtcaagaacaagggcggcggaggatccggcggtggtggttccggcggaggcggttctgaacctaagtcctccgacaagacccacacctgtcctccatgtcctgctccagaactgctcggcggaccttccgtgtttctgttcccacctaagccaaaggacaccctgatgatcagcagaacccctgaagtgacctgcgtggtggtggatgtgtctcacgaggaccccgaagtgaagttcaattggtacgtggacggcgtggaagtgcacaacgccaagaccaagcctagagaggaacagtacaactccacctacagagtggtgtccgtgctgaccgtgctgcaccaggattggctgaacggcaaagagtacaagtgcaaggtgtccaacaaggccctgcctgctcctatcgaaaagaccatctccaaggccaagggccagcctagggaaccccaggtttacacactgcctccatctcgggacgagctgaccaagaatcaggtgtccctgacctgtctggtcaagggcttctacccttccgatatcgccgtggaatgggagagcaatggccagcctgagaacaactacaagacaacccctcctgtgctggactccgacggctcattcttcctgtatagcaagctgacagtggacaagtcccggtggcagcagggcaacgtgttctcctgttctgtgatgcacgaggccctgcacaaccactacacccagaagagtctgtccttgagcccgggcggtggcggtggaagcggaggtggcggatctggtggcggaggtagtggcggaggcggatctcggtctaagcagagaaggcctcagggcctgcctaacaataccgcctcctggtttaccgctctgacccagcacggcaaagaggacctgaagttccctagaggacagggcgtgcccatcaacaccaactctagccctgacgaccagatcggctactacagacgggccaccagaagaatcagaggcggcgacggcaagatgaaggacctgtctcctcggtggtacttctactacctcggcaccggaccagaggctggattgccttatggcgccaacaaggacggcatcatctgggttgcaacagagggcgctctgaacacccctaaggaccacatcggcacccggaatcctgccaacaatgctgccattgtgctgcagctgccacagggcacaacactgcctaagggcttttacgccgagggctctagaggcggctctcaggcctcttccagatcctccagtagatcacgt